European Patent Specification EP 3 543 251 B1, published August 30, 2023. Title: A solid carrier comprising IgG binding peptide and a method for separating IgG. Applicant: Kagoshima University Daicel Corporation. The sequence listing filed with the application follows.

SEQUENCE LISTING (31 sequences)

SEQ ID NO: 1 - protein, 13 aa, Artificial
  Synthetic construct
  misc_feature (6)..(6): Xaa is arginine, lysine, leucine, asparagine, or derivative thereof
DCAYHXGELVWCT

SEQ ID NO: 2 - protein, 17 aa, Artificial
  Synthetic construct
  misc_feature (8)..(8): Xaa is arginine, lysine, leucine, asparagine, or derivative thereof
GPDCAYHXGELVWCTFH

SEQ ID NO: 3 - protein, 13 aa, Artificial
  Synthetic construct
  misc_feature (6)..(6): Xaa is arginine, lysine, leucine, asparagine, or derivative thereof
RCAYHXGELVWCS

SEQ ID NO: 4 - protein, 17 aa, Artificial
  Synthetic construct
  misc_feature (8)..(8): Xaa is arginine, lysine, leucine, asparagine, or derivative thereof
GPRCAYHXGELVWCSFH

SEQ ID NO: 5 - protein, 17 aa, Artificial
  Synthetic construct
  misc_feature (8)..(8): Xaa is arginine, lysine, leucine, asparagine, or derivative thereof
SPDCAYHXGELVWCTFH

SEQ ID NO: 6 - protein, 17 aa, Artificial
  Synthetic construct
  misc_feature (8)..(8): Xaa is arginine, lysine, leucine, asparagine, or derivative thereof
GDDCAYHXGELVWCTFH

SEQ ID NO: 7 - protein, 17 aa, Artificial
  Synthetic construct
  misc_feature (8)..(8): Xaa is arginine, lysine, leucine, asparagine, or derivative thereof
GPSCAYHXGELVWCTFH

SEQ ID NO: 8 - protein, 17 aa, Artificial
  Synthetic construct
  misc_feature (8)..(8): Xaa is arginine, lysine, leucine, asparagine, or derivative thereof
GPDCAYHXGELVWCSFH

SEQ ID NO: 9 - protein, 17 aa, Artificial
  Synthetic construct
  misc_feature (8)..(8): Xaa is arginine, lysine, leucine, asparagine, or derivative thereof
GPDCAYHXGELVWCTHH

SEQ ID NO: 10 - protein, 17 aa, Artificial
  Synthetic construct
  misc_feature (8)..(8): Xaa is arginine, lysine, leucine, asparagine, or derivative thereof
GPDCAYHXGELVWCTFY

SEQ ID NO: 11 - protein, 17 aa, Artificial
  Synthetic construct
  misc_feature (8)..(8): Xaa is arginine, lysine, leucine, asparagine, or derivative thereof
SPDCAYHXGELVWCTFY

SEQ ID NO: 12 - protein, 17 aa, Artificial
  Synthetic construct
  misc_feature (8)..(8): Xaa is arginine, lysine, leucine, asparagine, or derivative thereof
SDDCAYHXGELVWCTFY

SEQ ID NO: 13 - protein, 17 aa, Artificial
  Synthetic construct
  misc_feature (8)..(8): Xaa is arginine, lysine, leucine, asparagine, or derivative thereof
RGNCAYHXGQLVWCTYH

SEQ ID NO: 14 - protein, 17 aa, Artificial
  Synthetic construct
  misc_feature (2)..(2): Xaa is homoserine
  misc_feature (8)..(8): Xaa is arginine, lysine, leucine, asparagine, or derivative thereof
  misc_feature (16)..(16): Xaa is homoserine
GXDCAYHXGELVWCTXH

SEQ ID NO: 15 - protein, 13 aa, Artificial
  Synthetic construct
  misc_feature (6)..(6): Xaa is arginine, lysine, leucine, asparagine, or derivative thereof
DCTYHXGNLVWCT

SEQ ID NO: 16 - protein, 13 aa, Artificial
  Synthetic construct
  misc_feature (6)..(6): Xaa is arginine, lysine, leucine, asparagine, or derivative thereof
DCAYHXGNLVWCT

SEQ ID NO: 17 - protein, 13 aa, Artificial
  Synthetic construct
  misc_feature (6)..(6): Xaa is arginine, lysine, leucine, asparagine, or derivative thereof
DCTYHXGELVWCT

SEQ ID NO: 18 - protein, 13 aa, Artificial
  Synthetic construct
  misc_feature (6)..(6): Xaa is arginine, lysine, leucine, asparagine, or derivative thereof
DCAWHXGELVWCT

SEQ ID NO: 19 - protein, 13 aa, Artificial
  Synthetic construct
  misc_feature (6)..(6): Xaa is arginine, lysine, leucine, asparagine, or derivative thereof
DCTYTXGNLVWCT

SEQ ID NO: 20 - protein, 13 aa, Artificial
  Synthetic construct
  misc_feature (6)..(6): Xaa is arginine, lysine, leucine, asparagine, or derivative thereof
DCAYTXGNLVWCT

SEQ ID NO: 21 - protein, 13 aa, Artificial
  Synthetic construct
  misc_feature (6)..(6): Xaa is arginine, lysine, leucine, asparagine, or derivative thereof
DCSYTXGNLVWCT

SEQ ID NO: 22 - protein, 13 aa, Artificial
  Synthetic construct
  misc_feature (6)..(6): Xaa is arginine, lysine, leucine, asparagine, or derivative thereof
DCTWTXGNLVWCT

SEQ ID NO: 23 - protein, 13 aa, Artificial
  Synthetic construct
  misc_feature (6)..(6): Xaa is arginine, lysine, leucine, asparagine, or derivative thereof
DCTYHXGNLVWCT

SEQ ID NO: 24 - protein, 13 aa, Artificial
  Synthetic construct
  misc_feature (6)..(6): Xaa is arginine, lysine, leucine, asparagine, or derivative thereof
DCTYRXGNLVWCT

SEQ ID NO: 25 - protein, 13 aa, Artificial
  Synthetic construct
  misc_feature (6)..(6): Xaa is arginine, lysine, leucine, asparagine, or derivative thereof
DCTYSXGNLVWCT

SEQ ID NO: 26 - protein, 13 aa, Artificial
  Synthetic construct
  misc_feature (6)..(6): Xaa is arginine, lysine, leucine, asparagine, or derivative thereof
DCTYTXGNLVWCT

SEQ ID NO: 27 - protein, 13 aa, Artificial
  Synthetic construct
  misc_feature (6)..(6): Xaa is arginine, lysine, leucine, asparagine, or derivative thereof
DCTYTXGELVWCT

SEQ ID NO: 28 - protein, 13 aa, Artificial
  Synthetic construct
  misc_feature (6)..(6): Xaa is arginine, lysine, leucine, asparagine, or derivative thereof
DCTYTXGRLVWCT

SEQ ID NO: 29 - protein, 13 aa, Artificial
  Synthetic construct
  misc_feature (6)..(6): Xaa is arginine, lysine, leucine, asparagine, or derivative thereof
DCTYTXGDLVWCT

SEQ ID NO: 30 - protein, 13 aa, Artificial
  Synthetic construct
  misc_feature (6)..(6): Xaa is arginine, lysine, leucine, asparagine, or derivative thereof
DCTYTXGNLIWCT

SEQ ID NO: 31 - protein, 17 aa, Artificial
  Synthetic construct
GPDCAYHRGELVWCTFH